European Patent Application EP 4 606 893 A1, published August 27, 2025. Title: Novel CoA-acylating propionaldehyde dehydrogenase variant and uses thereof. Applicant: CJ CheilJedang Corporation. The sequence listing filed with the application follows.

SEQUENCE LISTING (46 sequences)

SEQ ID NO: 1 - protein, 464 aa, unidentified
MNTSELETLIRTILSEQLTTPAQTPVQPQGKGIFQSVSEAIDAAHQAFLRYQQCPLKTRSAIISAMRQELTPLLAPLAEESANETGMGNKEDKFLKNKAALDNTPGVEDLTTTALTGDGGMVLFEYSPFGVIGSVAPSTNPTETIINNSISMLAAGNSIYFSPHPGAKKVSLKLISLIEEIAFRCCGIRNLVVTVAEPTFEATQQMMAHPRIAVLAITGGPGIVAMGMKSGKKVIGAGAGNPPCIVDETADLVKAAEDIINGASFDYNLPCIAEKSLIVVESVAERLVQQMQTFGALLLSPADTDKLRAVCLPEGQANKKLVGKSPSAMLEAAGIAVPAKAPRLLIALVNADDPWVTSEQLMPMLPVVKVSDFDSALALALKVEEGLHHTAIMHSQNVSRLNLAARTLQTSIFVKNGPSYAGIGVGGEGFTTFTIATPTGEGTTSARTFARSRRCVLTNGFSIR

SEQ ID NO: 2 - DNA, 1395 bp, unidentified
  source 1..1395: mol_type = genomic DNA
atgaatacttctgaactcgaaaccctgattcgcaccattcttagcgagcaattaaccacgccggcgcaaacgccggtccagcctcagggcaaagggattttccagtccgtgagcgaggccatcgacgccgcgcaccaggcgttcttacgttatcagcagtgcccgctaaaaacccgcagcgccattatcagcgcgatgcgtcaggagctgacgccgctgctggcgcccctggcggaagagagcgccaatgaaacggggatgggcaacaaagaagataaatttctcaaaaacaaggctgcgctggacaacacgccgggcgtagaagatctcaccaccaccgcgctgaccggcgacggcggcatggtgctgtttgaatactcaccgtttggcgttatcggttcggtcgccccaagcaccaacccgacggaaaccatcatcaacaacagtatcagcatgctggcggcgggcaacagtatctactttagcccgcatccgggagcgaaaaaggtctctctgaagctgattagcctgattgaagagattgccttccgctgctgcggcatccgcaatctggtggtgaccgtggcggaacccaccttcgaagcgacccagcagatgatggcccacccgcgaatcgcagtactggccattaccggcggcccgggcattgtggcaatgggcatgaagagcggtaagaaggtgattggcgctggcgcgggtaacccgccctgcatcgttgatgaaacggcggacctggtgaaagcggcggaagatatcatcaacggcgcgtcattcgattacaacctgccctgcattgccgagaagagcctgatcgtagtggagagtgtcgccgaacgtctggtgcagcaaatgcaaaccttcggcgcgctgctgttaagccctgccgataccgacaaactccgcgccgtctgcctgcctgaaggccaggcgaataaaaaactggtcggcaagagcccatcggccatgctggaagccgccgggatcgctgtccctgcaaaagcgccgcgtctgctgattgcgctggttaacgctgacgatccgtgggtcaccagcgaacagttgatgccgatgctgccagtggtaaaagtcagcgatttcgatagcgcgctggcgctggccctgaaggttgaagaggggctgcatcataccgccattatgcactcgcagaacgtgtcacgcctgaacctcgcggcccgcacgctgcaaacctcgatattcgtcaaaaacggcccctcttatgccgggatcggcgtcggcggcgaaggctttaccaccttcactatcgccacaccaaccggtgaagggaccacgtcagcgcgtacttttgcccgttcccggcgctgcgtactgaccaacggcttttctattcgctaa

SEQ ID NO: 3 - protein, 464 aa, synthetic construct
MNTSELETLIRTILSEQLTTPAQTPVQPQGKGIFQSVSEAIDAAHQAFLRYQQCPLKTRSAIISAMRQELTPLLAPLAEESANETGMGNKEDKFLKNKAALDNTPGVEDLTTTALTGDGGMVLFEYSPFGVIGSVAPSTNPTETIINNSISMLAAGNSIYFSPHPGAKKVSLKLISLIEEIAFRCCGIRNLVVTVAEPTFEATQQMMAHPRIAVLAITGGPGIVAMGMKSGKKVIGAGAGNPPCIVDETADLVKAAEDIINGASFDYNLPCTAEKSLIVVESVAERLVQQMQTFGALLLSPADTDKLRAVCLPEGQANKKLVGKSPSAMLEAAGIAVPAKAPRLLIALVNADDPWVTSEQLMPMLPVVKVSDFDSALALALKVEEGLHHTAIMHSQNVSRLNLAARTLQTSIFVKNGPSYAGIGVGGEGFTTFTIATPTGEGTTSARTFARSRRCVLTNGFSIR

SEQ ID NO: 4 - protein, 464 aa, synthetic construct
MNTSELETLIRTILSEQLTTPAQTPVQPQGKGIFQSVSEAIDAAHQAFLRYQQCPLKTRSAIISAMRQELTPLLAPLAEESANETGMGNKEDKFLKNKAALDNTPGVEDLTTTALTGDGGMVLFEYSPFGVIGSVAPSTNPTETIINNSISMLAAGNSIYFSPHPGAKKVSLKLISLIEEIAFRCCGIRNLVVTVAEPTFEATQQMMAHPRIAVLAITGGPGIVAMGMKSGKKVIGAGAGNPPCIVDETADLVKAAEDIINGASFDYNLPCVAEKSLIVVESVAERLVQQMQTFGALLLSPADTDKLRAVCLPEGQANKKLVGKSPSAMLEAAGIAVPAKAPRLLIALVNADDPWVTSEQLMPMLPVVKVSDFDSALALALKVEEGLHHTAIMHSQNVSRLNLAARTLQTSIFVKNGPSYAGIGVGGEGFTTFTIATPTGEGTTSARTFARSRRCVLTNGFSIR

SEQ ID NO: 5 - protein, 464 aa, synthetic construct
MNTSELETLIRTILSEQLTTPAQTPVQPQGKGIFQSVSEAIDAAHQAFLRYQQCPLKTRSAIISAMRQELTPLLAPLAEESANETGMGNKEDKFLKNKAALDNTPGVEDLTTTALTGDGGMVLFEYSPFGVIGSVAPSTNPTETIINNSISMLAAGNSIYFSPHPGAKKVSLKLISLIEEIAFRCCGIRNLVVTVAEPTFEATQQMMAHPRIAVLAITGGPGIVAMGMKSGKKVIGAGAGNPPCIVDETADLVKAAEDIINGASFDYNLPCYAEKSLIVVESVAERLVQQMQTFGALLLSPADTDKLRAVCLPEGQANKKLVGKSPSAMLEAAGIAVPAKAPRLLIALVNADDPWVTSEQLMPMLPVVKVSDFDSALALALKVEEGLHHTAIMHSQNVSRLNLAARTLQTSIFVKNGPSYAGIGVGGEGFTTFTIATPTGEGTTSARTFARSRRCVLTNGFSIR

SEQ ID NO: 6 - protein, 464 aa, synthetic construct
MNTSELETLIRTILSEQLTTPAQTPVQPQGKGIFQSVSEAIDAAHQAFLRYQQCPLKTRSAIISAMRQELTPLLAPLAEESANETGMGNKEDKFLKNKAALDNTPGVEDLTTTALTGDGGMVLFEYSPFGVIGSVAPSTNPTETIINNSISMLAAGNSIYFSPHPGAKKVSLKLISLIEEIAFRCCGIRNLVVTVAEPTFEATQQMMAHPRIAVLAITGGPGIVAMGMKSGKKVIGAGAGNPPCIVDETADLVKAAEDIINGASFDYNLPCNAEKSLIVVESVAERLVQQMQTFGALLLSPADTDKLRAVCLPEGQANKKLVGKSPSAMLEAAGIAVPAKAPRLLIALVNADDPWVTSEQLMPMLPVVKVSDFDSALALALKVEEGLHHTAIMHSQNVSRLNLAARTLQTSIFVKNGPSYAGIGVGGEGFTTFTIATPTGEGTTSARTFARSRRCVLTNGFSIR

SEQ ID NO: 7 - protein, 464 aa, synthetic construct
MNTSELETLIRTILSEQLTTPAQTPVQPQGKGIFQSVSEAIDAAHQAFLRYQQCPLKTRSAIISAMRQELTPLLAPLAEESANETGMGNKEDKFLKNKAALDNTPGVEDLTTTALTGDGGMVLFEYSPFGVIGSVAPSTNPTETIINNSISMLAAGNSIYFSPHPGAKKVSLKLISLIEEIAFRCCGIRNLVVTVAEPTFEATQQMMAHPRIAVLAITGGPGIVAMGMKSGKKVIGAGAGNPPCIVDETADLVKAAEDIINGASFDYNLPCQAEKSLIVVESVAERLVQQMQTFGALLLSPADTDKLRAVCLPEGQANKKLVGKSPSAMLEAAGIAVPAKAPRLLIALVNADDPWVTSEQLMPMLPVVKVSDFDSALALALKVEEGLHHTAIMHSQNVSRLNLAARTLQTSIFVKNGPSYAGIGVGGEGFTTFTIATPTGEGTTSARTFARSRRCVLTNGFSIR

SEQ ID NO: 8 - DNA, 44 bp, synthetic construct
  source 1..44: mol_type = other DNA
ctaggattcaggaggtttttatgaatacttctgaactcgaaacc

SEQ ID NO: 9 - DNA, 45 bp, synthetic construct
  source 1..45: mol_type = other DNA
ctcaaaagggtcgacaaatcttagcgaatagaaaagccgttggtc

SEQ ID NO: 10 - DNA, 26 bp, synthetic construct
  source 1..26: mol_type = other DNA
gatttgtcgacccttttgagccgatg

SEQ ID NO: 11 - DNA, 26 bp, synthetic construct
  source 1..26: mol_type = other DNA
aaaaacctcctgaatcctagaggatc

SEQ ID NO: 12 - DNA, 22 bp, synthetic construct
  source 1..22: mol_type = other DNA
atatcgccggtgtgatcaaccc

SEQ ID NO: 13 - DNA, 29 bp, synthetic construct
  source 1..29: mol_type = other DNA
tgcgctcaacgttgatcgcgtaatcggcg

SEQ ID NO: 14 - DNA, 25 bp, synthetic construct
  source 1..25: mol_type = other DNA
gcagggcaggttgtaatcgaatgac

SEQ ID NO: 15 - DNA, 45 bp, synthetic construct
  source 1..45: mol_type = other DNA
tcgattacaacctgccctgcggtgccgagaagagcctgatcgtag

SEQ ID NO: 16 - DNA, 45 bp, synthetic construct
  source 1..45: mol_type = other DNA
tcgattacaacctgccctgcgcggccgagaagagcctgatcgtag

SEQ ID NO: 17 - DNA, 45 bp, synthetic construct
  source 1..45: mol_type = other DNA
tcgattacaacctgccctgcgtggccgagaagagcctgatcgtag

SEQ ID NO: 18 - DNA, 45 bp, synthetic construct
  source 1..45: mol_type = other DNA
tcgattacaacctgccctgcctggccgagaagagcctgatcgtag

SEQ ID NO: 19 - DNA, 45 bp, synthetic construct
  source 1..45: mol_type = other DNA
tcgattacaacctgccctgcatggccgagaagagcctgatcgtag

SEQ ID NO: 20 - DNA, 45 bp, synthetic construct
  source 1..45: mol_type = other DNA
tcgattacaacctgccctgctttgccgagaagagcctgatcgtag

SEQ ID NO: 21 - DNA, 45 bp, synthetic construct
  source 1..45: mol_type = other DNA
tcgattacaacctgccctgctgggccgagaagagcctgatcgtag

SEQ ID NO: 22 - DNA, 45 bp, synthetic construct
  source 1..45: mol_type = other DNA
tcgattacaacctgccctgcccggccgagaagagcctgatcgtag

SEQ ID NO: 23 - DNA, 45 bp, synthetic construct
  source 1..45: mol_type = other DNA
tcgattacaacctgccctgcagcgccgagaagagcctgatcgtag

SEQ ID NO: 24 - DNA, 45 bp, synthetic construct
  source 1..45: mol_type = other DNA
tcgattacaacctgccctgctgcgccgagaagagcctgatcgtag

SEQ ID NO: 25 - DNA, 45 bp, synthetic construct
  source 1..45: mol_type = other DNA
tcgattacaacctgccctgctatgccgagaagagcctgatcgtag

SEQ ID NO: 26 - DNA, 45 bp, synthetic construct
  source 1..45: mol_type = other DNA
tcgattacaacctgccctgcaacgccgagaagagcctgatcgtag

SEQ ID NO: 27 - DNA, 45 bp, synthetic construct
  source 1..45: mol_type = other DNA
tcgattacaacctgccctgccaggccgagaagagcctgatcgtag

SEQ ID NO: 28 - DNA, 45 bp, synthetic construct
  source 1..45: mol_type = other DNA
tcgattacaacctgccctgcgatgccgagaagagcctgatcgtag

SEQ ID NO: 29 - DNA, 45 bp, synthetic construct
  source 1..45: mol_type = other DNA
tcgattacaacctgccctgcgaagccgagaagagcctgatcgtag

SEQ ID NO: 30 - DNA, 45 bp, synthetic construct
  source 1..45: mol_type = other DNA
tcgattacaacctgccctgcaaagccgagaagagcctgatcgtag

SEQ ID NO: 31 - DNA, 45 bp, synthetic construct
  source 1..45: mol_type = other DNA
tcgattacaacctgccctgccgtgccgagaagagcctgatcgtag

SEQ ID NO: 32 - DNA, 45 bp, synthetic construct
  source 1..45: mol_type = other DNA
tcgattacaacctgccctgccatgccgagaagagcctgatcgtag

SEQ ID NO: 33 - protein, 464 aa, synthetic construct
MNTSELETLIRTILSEQLTTPAQTPVQPQGKGIFQSVSEAIDAAHQAFLRYQQCPLKTRSAIISAMRQELTPLLAPLAEESANETGMGNKEDKFLKNKAALDNTPGVEDLTTTALTGDGGMVLFEYSPFGVIGSVAPSTNPTETIINNSISMLAAGNSIYFSPHPGAKKVSLKLISLIEEIAFRCCGIRNLVVTVAEPTFEATQQMMAHPRIAVLAITGGPGIVAMGMKSGKKVIGAGAGNPPCIVDETADLVKAAEDIINGASFDYNLPCGAEKSLIVVESVAERLVQQMQTFGALLLSPADTDKLRAVCLPEGQANKKLVGKSPSAMLEAAGIAVPAKAPRLLIALVNADDPWVTSEQLMPMLPVVKVSDFDSALALALKVEEGLHHTAIMHSQNVSRLNLAARTLQTSIFVKNGPSYAGIGVGGEGFTTFTIATPTGEGTTSARTFARSRRCVLTNGFSIR

SEQ ID NO: 34 - protein, 464 aa, synthetic construct
MNTSELETLIRTILSEQLTTPAQTPVQPQGKGIFQSVSEAIDAAHQAFLRYQQCPLKTRSAIISAMRQELTPLLAPLAEESANETGMGNKEDKFLKNKAALDNTPGVEDLTTTALTGDGGMVLFEYSPFGVIGSVAPSTNPTETIINNSISMLAAGNSIYFSPHPGAKKVSLKLISLIEEIAFRCCGIRNLVVTVAEPTFEATQQMMAHPRIAVLAITGGPGIVAMGMKSGKKVIGAGAGNPPCIVDETADLVKAAEDIINGASFDYNLPCAAEKSLIVVESVAERLVQQMQTFGALLLSPADTDKLRAVCLPEGQANKKLVGKSPSAMLEAAGIAVPAKAPRLLIALVNADDPWVTSEQLMPMLPVVKVSDFDSALALALKVEEGLHHTAIMHSQNVSRLNLAARTLQTSIFVKNGPSYAGIGVGGEGFTTFTIATPTGEGTTSARTFARSRRCVLTNGFSIR

SEQ ID NO: 35 - protein, 464 aa, synthetic construct
MNTSELETLIRTILSEQLTTPAQTPVQPQGKGIFQSVSEAIDAAHQAFLRYQQCPLKTRSAIISAMRQELTPLLAPLAEESANETGMGNKEDKFLKNKAALDNTPGVEDLTTTALTGDGGMVLFEYSPFGVIGSVAPSTNPTETIINNSISMLAAGNSIYFSPHPGAKKVSLKLISLIEEIAFRCCGIRNLVVTVAEPTFEATQQMMAHPRIAVLAITGGPGIVAMGMKSGKKVIGAGAGNPPCIVDETADLVKAAEDIINGASFDYNLPCLAEKSLIVVESVAERLVQQMQTFGALLLSPADTDKLRAVCLPEGQANKKLVGKSPSAMLEAAGIAVPAKAPRLLIALVNADDPWVTSEQLMPMLPVVKVSDFDSALALALKVEEGLHHTAIMHSQNVSRLNLAARTLQTSIFVKNGPSYAGIGVGGEGFTTFTIATPTGEGTTSARTFARSRRCVLTNGFSIR

SEQ ID NO: 36 - protein, 464 aa, synthetic construct
MNTSELETLIRTILSEQLTTPAQTPVQPQGKGIFQSVSEAIDAAHQAFLRYQQCPLKTRSAIISAMRQELTPLLAPLAEESANETGMGNKEDKFLKNKAALDNTPGVEDLTTTALTGDGGMVLFEYSPFGVIGSVAPSTNPTETIINNSISMLAAGNSIYFSPHPGAKKVSLKLISLIEEIAFRCCGIRNLVVTVAEPTFEATQQMMAHPRIAVLAITGGPGIVAMGMKSGKKVIGAGAGNPPCIVDETADLVKAAEDIINGASFDYNLPCMAEKSLIVVESVAERLVQQMQTFGALLLSPADTDKLRAVCLPEGQANKKLVGKSPSAMLEAAGIAVPAKAPRLLIALVNADDPWVTSEQLMPMLPVVKVSDFDSALALALKVEEGLHHTAIMHSQNVSRLNLAARTLQTSIFVKNGPSYAGIGVGGEGFTTFTIATPTGEGTTSARTFARSRRCVLTNGFSIR

SEQ ID NO: 37 - protein, 464 aa, synthetic construct
MNTSELETLIRTILSEQLTTPAQTPVQPQGKGIFQSVSEAIDAAHQAFLRYQQCPLKTRSAIISAMRQELTPLLAPLAEESANETGMGNKEDKFLKNKAALDNTPGVEDLTTTALTGDGGMVLFEYSPFGVIGSVAPSTNPTETIINNSISMLAAGNSIYFSPHPGAKKVSLKLISLIEEIAFRCCGIRNLVVTVAEPTFEATQQMMAHPRIAVLAITGGPGIVAMGMKSGKKVIGAGAGNPPCIVDETADLVKAAEDIINGASFDYNLPCFAEKSLIVVESVAERLVQQMQTFGALLLSPADTDKLRAVCLPEGQANKKLVGKSPSAMLEAAGIAVPAKAPRLLIALVNADDPWVTSEQLMPMLPVVKVSDFDSALALALKVEEGLHHTAIMHSQNVSRLNLAARTLQTSIFVKNGPSYAGIGVGGEGFTTFTIATPTGEGTTSARTFARSRRCVLTNGFSIR

SEQ ID NO: 38 - protein, 464 aa, synthetic construct
MNTSELETLIRTILSEQLTTPAQTPVQPQGKGIFQSVSEAIDAAHQAFLRYQQCPLKTRSAIISAMRQELTPLLAPLAEESANETGMGNKEDKFLKNKAALDNTPGVEDLTTTALTGDGGMVLFEYSPFGVIGSVAPSTNPTETIINNSISMLAAGNSIYFSPHPGAKKVSLKLISLIEEIAFRCCGIRNLVVTVAEPTFEATQQMMAHPRIAVLAITGGPGIVAMGMKSGKKVIGAGAGNPPCIVDETADLVKAAEDIINGASFDYNLPCWAEKSLIVVESVAERLVQQMQTFGALLLSPADTDKLRAVCLPEGQANKKLVGKSPSAMLEAAGIAVPAKAPRLLIALVNADDPWVTSEQLMPMLPVVKVSDFDSALALALKVEEGLHHTAIMHSQNVSRLNLAARTLQTSIFVKNGPSYAGIGVGGEGFTTFTIATPTGEGTTSARTFARSRRCVLTNGFSIR

SEQ ID NO: 39 - protein, 464 aa, synthetic construct
MNTSELETLIRTILSEQLTTPAQTPVQPQGKGIFQSVSEAIDAAHQAFLRYQQCPLKTRSAIISAMRQELTPLLAPLAEESANETGMGNKEDKFLKNKAALDNTPGVEDLTTTALTGDGGMVLFEYSPFGVIGSVAPSTNPTETIINNSISMLAAGNSIYFSPHPGAKKVSLKLISLIEEIAFRCCGIRNLVVTVAEPTFEATQQMMAHPRIAVLAITGGPGIVAMGMKSGKKVIGAGAGNPPCIVDETADLVKAAEDIINGASFDYNLPCPAEKSLIVVESVAERLVQQMQTFGALLLSPADTDKLRAVCLPEGQANKKLVGKSPSAMLEAAGIAVPAKAPRLLIALVNADDPWVTSEQLMPMLPVVKVSDFDSALALALKVEEGLHHTAIMHSQNVSRLNLAARTLQTSIFVKNGPSYAGIGVGGEGFTTFTIATPTGEGTTSARTFARSRRCVLTNGFSIR

SEQ ID NO: 40 - protein, 464 aa, synthetic construct
MNTSELETLIRTILSEQLTTPAQTPVQPQGKGIFQSVSEAIDAAHQAFLRYQQCPLKTRSAIISAMRQELTPLLAPLAEESANETGMGNKEDKFLKNKAALDNTPGVEDLTTTALTGDGGMVLFEYSPFGVIGSVAPSTNPTETIINNSISMLAAGNSIYFSPHPGAKKVSLKLISLIEEIAFRCCGIRNLVVTVAEPTFEATQQMMAHPRIAVLAITGGPGIVAMGMKSGKKVIGAGAGNPPCIVDETADLVKAAEDIINGASFDYNLPCSAEKSLIVVESVAERLVQQMQTFGALLLSPADTDKLRAVCLPEGQANKKLVGKSPSAMLEAAGIAVPAKAPRLLIALVNADDPWVTSEQLMPMLPVVKVSDFDSALALALKVEEGLHHTAIMHSQNVSRLNLAARTLQTSIFVKNGPSYAGIGVGGEGFTTFTIATPTGEGTTSARTFARSRRCVLTNGFSIR

SEQ ID NO: 41 - protein, 464 aa, synthetic construct
MNTSELETLIRTILSEQLTTPAQTPVQPQGKGIFQSVSEAIDAAHQAFLRYQQCPLKTRSAIISAMRQELTPLLAPLAEESANETGMGNKEDKFLKNKAALDNTPGVEDLTTTALTGDGGMVLFEYSPFGVIGSVAPSTNPTETIINNSISMLAAGNSIYFSPHPGAKKVSLKLISLIEEIAFRCCGIRNLVVTVAEPTFEATQQMMAHPRIAVLAITGGPGIVAMGMKSGKKVIGAGAGNPPCIVDETADLVKAAEDIINGASFDYNLPCCAEKSLIVVESVAERLVQQMQTFGALLLSPADTDKLRAVCLPEGQANKKLVGKSPSAMLEAAGIAVPAKAPRLLIALVNADDPWVTSEQLMPMLPVVKVSDFDSALALALKVEEGLHHTAIMHSQNVSRLNLAARTLQTSIFVKNGPSYAGIGVGGEGFTTFTIATPTGEGTTSARTFARSRRCVLTNGFSIR

SEQ ID NO: 42 - protein, 464 aa, synthetic construct
MNTSELETLIRTILSEQLTTPAQTPVQPQGKGIFQSVSEAIDAAHQAFLRYQQCPLKTRSAIISAMRQELTPLLAPLAEESANETGMGNKEDKFLKNKAALDNTPGVEDLTTTALTGDGGMVLFEYSPFGVIGSVAPSTNPTETIINNSISMLAAGNSIYFSPHPGAKKVSLKLISLIEEIAFRCCGIRNLVVTVAEPTFEATQQMMAHPRIAVLAITGGPGIVAMGMKSGKKVIGAGAGNPPCIVDETADLVKAAEDIINGASFDYNLPCDAEKSLIVVESVAERLVQQMQTFGALLLSPADTDKLRAVCLPEGQANKKLVGKSPSAMLEAAGIAVPAKAPRLLIALVNADDPWVTSEQLMPMLPVVKVSDFDSALALALKVEEGLHHTAIMHSQNVSRLNLAARTLQTSIFVKNGPSYAGIGVGGEGFTTFTIATPTGEGTTSARTFARSRRCVLTNGFSIR

SEQ ID NO: 43 - protein, 464 aa, synthetic construct
MNTSELETLIRTILSEQLTTPAQTPVQPQGKGIFQSVSEAIDAAHQAFLRYQQCPLKTRSAIISAMRQELTPLLAPLAEESANETGMGNKEDKFLKNKAALDNTPGVEDLTTTALTGDGGMVLFEYSPFGVIGSVAPSTNPTETIINNSISMLAAGNSIYFSPHPGAKKVSLKLISLIEEIAFRCCGIRNLVVTVAEPTFEATQQMMAHPRIAVLAITGGPGIVAMGMKSGKKVIGAGAGNPPCIVDETADLVKAAEDIINGASFDYNLPCEAEKSLIVVESVAERLVQQMQTFGALLLSPADTDKLRAVCLPEGQANKKLVGKSPSAMLEAAGIAVPAKAPRLLIALVNADDPWVTSEQLMPMLPVVKVSDFDSALALALKVEEGLHHTAIMHSQNVSRLNLAARTLQTSIFVKNGPSYAGIGVGGEGFTTFTIATPTGEGTTSARTFARSRRCVLTNGFSIR

SEQ ID NO: 44 - protein, 464 aa, synthetic construct
MNTSELETLIRTILSEQLTTPAQTPVQPQGKGIFQSVSEAIDAAHQAFLRYQQCPLKTRSAIISAMRQELTPLLAPLAEESANETGMGNKEDKFLKNKAALDNTPGVEDLTTTALTGDGGMVLFEYSPFGVIGSVAPSTNPTETIINNSISMLAAGNSIYFSPHPGAKKVSLKLISLIEEIAFRCCGIRNLVVTVAEPTFEATQQMMAHPRIAVLAITGGPGIVAMGMKSGKKVIGAGAGNPPCIVDETADLVKAAEDIINGASFDYNLPCKAEKSLIVVESVAERLVQQMQTFGALLLSPADTDKLRAVCLPEGQANKKLVGKSPSAMLEAAGIAVPAKAPRLLIALVNADDPWVTSEQLMPMLPVVKVSDFDSALALALKVEEGLHHTAIMHSQNVSRLNLAARTLQTSIFVKNGPSYAGIGVGGEGFTTFTIATPTGEGTTSARTFARSRRCVLTNGFSIR

SEQ ID NO: 45 - protein, 464 aa, synthetic construct
MNTSELETLIRTILSEQLTTPAQTPVQPQGKGIFQSVSEAIDAAHQAFLRYQQCPLKTRSAIISAMRQELTPLLAPLAEESANETGMGNKEDKFLKNKAALDNTPGVEDLTTTALTGDGGMVLFEYSPFGVIGSVAPSTNPTETIINNSISMLAAGNSIYFSPHPGAKKVSLKLISLIEEIAFRCCGIRNLVVTVAEPTFEATQQMMAHPRIAVLAITGGPGIVAMGMKSGKKVIGAGAGNPPCIVDETADLVKAAEDIINGASFDYNLPCRAEKSLIVVESVAERLVQQMQTFGALLLSPADTDKLRAVCLPEGQANKKLVGKSPSAMLEAAGIAVPAKAPRLLIALVNADDPWVTSEQLMPMLPVVKVSDFDSALALALKVEEGLHHTAIMHSQNVSRLNLAARTLQTSIFVKNGPSYAGIGVGGEGFTTFTIATPTGEGTTSARTFARSRRCVLTNGFSIR

SEQ ID NO: 46 - protein, 464 aa, synthetic construct
MNTSELETLIRTILSEQLTTPAQTPVQPQGKGIFQSVSEAIDAAHQAFLRYQQCPLKTRSAIISAMRQELTPLLAPLAEESANETGMGNKEDKFLKNKAALDNTPGVEDLTTTALTGDGGMVLFEYSPFGVIGSVAPSTNPTETIINNSISMLAAGNSIYFSPHPGAKKVSLKLISLIEEIAFRCCGIRNLVVTVAEPTFEATQQMMAHPRIAVLAITGGPGIVAMGMKSGKKVIGAGAGNPPCIVDETADLVKAAEDIINGASFDYNLPCHAEKSLIVVESVAERLVQQMQTFGALLLSPADTDKLRAVCLPEGQANKKLVGKSPSAMLEAAGIAVPAKAPRLLIALVNADDPWVTSEQLMPMLPVVKVSDFDSALALALKVEEGLHHTAIMHSQNVSRLNLAARTLQTSIFVKNGPSYAGIGVGGEGFTTFTIATPTGEGTTSARTFARSRRCVLTNGFSIR